European Patent Application EP 4 295 843 A1, published December 27, 2023. Title: Compositions comprising amino acids for use in the prevention and/or treatment of intestinal diseases. Applicant: Professional Dietetics S.p.A. Application EP. The sequence listing filed with the application follows.

SEQUENCE LISTING (22 sequences)

SEQ ID NO: 1 - DNA, 20 bp, synthetic construct
  source 1..20: mol_type = other DNA
ccgttggcatgaagtgtatg

SEQ ID NO: 2 - DNA, 20 bp, synthetic construct
  source 1..20: mol_type = other DNA
ccagtgaagagagcctgacc

SEQ ID NO: 3 - DNA, 20 bp, synthetic construct
  source 1..20: mol_type = other DNA
aaggtgtacgactcgctgct

SEQ ID NO: 4 - DNA, 20 bp, synthetic construct
  source 1..20: mol_type = other DNA
agtcccggataatggtgttg

SEQ ID NO: 5 - DNA, 21 bp, synthetic construct
  source 1..21: mol_type = other DNA
gtctgcctgcatctcctctgt

SEQ ID NO: 6 - DNA, 20 bp, synthetic construct
  source 1..20: mol_type = other DNA
cctctaaacccgtccatcca

SEQ ID NO: 7 - DNA, 20 bp, synthetic construct
  source 1..20: mol_type = other DNA
ccagaaggcattgaaggaga

SEQ ID NO: 8 - DNA, 20 bp, synthetic construct
  source 1..20: mol_type = other DNA
ccagaaggcattgaaggaga

SEQ ID NO: 9 - DNA, 21 bp, synthetic construct
  source 1..21: mol_type = other DNA
cgttgtgccagcgactaaaaa

SEQ ID NO: 10 - DNA, 18 bp, synthetic construct
  source 1..18: mol_type = other DNA
ttccgcccaaagagacca

SEQ ID NO: 11 - DNA, 20 bp, synthetic construct
  source 1..20: mol_type = other DNA
tggaccgagagagtttccct

SEQ ID NO: 12 - DNA, 20 bp, synthetic construct
  source 1..20: mol_type = other DNA
cccttgtacgtggtgggatt

SEQ ID NO: 13 - DNA, 21 bp, synthetic construct
  source 1..21: mol_type = other DNA
ggctgagaacgggaagcttgt

SEQ ID NO: 14 - DNA, 20 bp, synthetic construct
  source 1..20: mol_type = other DNA
ccagcatcgccccacttgat

SEQ ID NO: 15 - DNA, 20 bp, synthetic construct
  source 1..20: mol_type = other DNA
gaagccaaacctctgtgagc

SEQ ID NO: 16 - DNA, 20 bp, synthetic construct
  source 1..20: mol_type = other DNA
gaagacatcgtctggggtgt

SEQ ID NO: 17 - DNA, 20 bp, synthetic construct
  source 1..20: mol_type = other DNA
agctgctgaagaggcaagag

SEQ ID NO: 18 - DNA, 20 bp, synthetic construct
  source 1..20: mol_type = other DNA
ttcccctaaaccaagcacac

SEQ ID NO: 19 - DNA, 18 bp, synthetic construct
  source 1..18: mol_type = other DNA
agattggggtcgggtcac

SEQ ID NO: 20 - DNA, 21 bp, synthetic construct
  source 1..21: mol_type = other DNA
gacaacttgccaagacagatg

SEQ ID NO: 21 - DNA, 22 bp, synthetic construct
  source 1..22: mol_type = other DNA
gaatgatggttggtatggtgcg

SEQ ID NO: 22 - DNA, 22 bp, synthetic construct
  source 1..22: mol_type = other DNA
tcagaagtgtgtctactgtccg